European Patent Application EP 4 163 369 A1, published April 12, 2023. Title: Use of Mixtures of Polyviinylpyrrolidone and Ammonium Sulfate in the Isolation of Nucleic Acids. Applicant: Axagarius GmbH & Co. KG. The sequence listing filed with the application follows.

SEQUENCE LISTING (12 sequences)

SEQ ID NO: 1 - DNA, 22 bp, arteficial
  misc_feature: CDV forward primer
ctgtcrgtaatcgagrattcga

SEQ ID NO: 2 - DNA, 23 bp, arteficial
  misc_feature: CDV reverse primer
gccgaaagaatatccccagttag

SEQ ID NO: 3 - DNA, 24 bp, arteficial
  misc_feature: CDV probe
atcttcgccagartcytcagtgct

SEQ ID NO: 4 - DNA, 22 bp, arteficial
  misc_feature: BTV forward primer
gttacgcattaccgaggttgtg

SEQ ID NO: 5 - DNA, 21 bp, arteficial
  misc_feature: BTV reverse primer
gatcatgtgtgaacgccttcg

SEQ ID NO: 6 - DNA, 24 bp, arteficial
  misc_feature: BTV probe
aacggctcacaccgacgatccagc

SEQ ID NO: 7 - DNA, 20 bp, arteficial
  misc_feature: PEV forward primer
gaatgcggctaatccyaacc

SEQ ID NO: 8 - DNA, 20 bp, arteficial
  misc_feature: PEV reverse primer
gttgtcaccataagcagcca

SEQ ID NO: 9 - DNA, 22 bp, arteficial
  misc_feature: PEV probe
acccaaagtagtcggttccgcc

SEQ ID NO: 10 - DNA, 22 bp, arteficial
  misc_feature: POX forward primer
gccagagatatcatagccgctc

SEQ ID NO: 11 - DNA, 29 bp, arteficial
  misc_feature: POX reverse primer
caacgactaactaatttggaaaaaaagat

SEQ ID NO: 12 - DNA, 34 bp, arteficial
  misc_feature: POX probe
ttttccaacctaaatagaacttcatcgttgcgtt